European Patent Application EP 4 778 533 A2, published July 22, 2026. Title: Bispecific Antibody Targeting IL-1R1 and NLPR3. Applicant: University of Ulster. Application EP. The sequence listing filed with the application follows.

SEQUENCE LISTING (69 sequences)

SEQ ID NO: 1 - protein, 550 aa, unidentified
  REGION 1..550: note = Synthetic
MKVLLRLICFIALLISSLEADKCKEREEKIILVSSANEIDVRPCPLNPNEHKGTITWYKDDSKTPVSTEQASRIHQHKEKLWFVPAKVEDSGHYYCVVRNSSYCLRIKISAKFVENEPNLCYNAQAIFKQKLPVAGDGGLVCPYMEFFKNENNELPKLQWYKDCKPLLLDNIHFSGVKDRLIVMNVAEKHRGNYTCHASYTYLGKQYPITRVIEFITLEENKPTRPVIVSPANETMEVDLGSQIQLICNVTGQLSDIAYWKWNGSVIDEDDPVLGEDYYSVENPANKRRSTLITVLNISEIESRFYKHPFTCFAKNTHGIDAAYIQLIYPVTNFQKLEGGPSVFIFPPNIKDVLMISLTPKVTCVVVDVSEDDPDVQISWFVNNVEVHTAQTQTHREDYNSTIRVVSHLPIQHQDWMSGKEFKCKVNNKDLPSPIERTISKPKGLVRAPQVYTLPPPAEQLSRKDVSLTCLVVGFNPGDISVEWTSNGHTEENYKDTAPVLDSDGSYFIYSKLNMKTSKWEKTDSFSCNVRHEGLKNYYLKKTISRSPGK

SEQ ID NO: 2 - protein, 151 aa, unidentified
  REGION 1..151: note = Synthetic
MEWSCVMLFLMAAAQSIQAQIQLVQSGPELRKPGETVRISCKASGYPFTTAGLQWVQKMSGKGLKWIGWMNTQSEVPKYAEEFKGRIAFSLETAASTAYLQINNLKTEDTATYFCAKSVYFNWRYFDVWGAGTTVTVSSAKTTPPPVYPLA

SEQ ID NO: 3 - protein, 153 aa, unidentified
  REGION 1..153: note = Synthetic
VHMECSCVMLFLMAAAQSIQAQIQLVQSGPELRKPGETVRISRKASGYPFTTAGLQWVQKMSGKGLKWIGWMNTQSEVPKYAEEFKGRIAFSLETAASTAYLQINNLKTEDTATYFCAKSVYFNWRYFDVWGAGTTVTVSSAKTTPPSVFPLA

SEQ ID NO: 4 - protein, 153 aa, unidentified
  REGION 1..153: note = Synthetic
VHMGWSWVMLFLMAAAQSIQAQIQLVQSGPELRKPGETVRISCKASGYPFTTAGLQWVQKMSGKGLKWIGWMNTQSEVPKYAEEFKGRIAFSLETAASTAYLQINNLKTEDTATYFCAKSVYFNWRYFDVWGAGTTVTVSSAKTTPPPVYPLA

SEQ ID NO: 5 - protein, 151 aa, unidentified
  REGION 1..151: note = Synthetic
MGWVWNLLFLMAAAQSIQAQIQLVQSGPELRKPGETVRISCKASGYPFTTAGLQWVQKMSGKGLKWIGWMNTQSEVPKYAEEFKGRIAFSLETAASTAYLQINNLKTEDTATYFCAKSVYFNWRYFDVWGAGTTVTVSSAKTTPPPVYPLV

SEQ ID NO: 6 - protein, 151 aa, unidentified
  REGION 1..151: note = Synthetic
MGWVWTLPFLMAAAQSIQAQIQLVQSGPELRKPGETVRISCKASGYPFTTAGLQWVQKMSGKGLKWIGWMNTQSEVPKYAEEFKGRIAFSLETAASTAYLQINNLKTEDTATYFCAKSVYFNWRYFDVWGAGTTVTVSSAKTTPPPVYPLV

SEQ ID NO: 7 - protein, 151 aa, unidentified
  REGION 1..151: note = Synthetic
MGWVWNLPFLMAAAQSIQAQIQLVQSGPELRKPGETVRISCKASGYPFTTAGLQWVQKMSGKGLKWIGWMNTQSEVPKYAEEFKGRIAFSLETAASTAYLQINNLKTEDTATYFCAKSVYFNWRYFDVWGAGTTVTVSSAKTTPPPVYPLA

SEQ ID NO: 8 - protein, 151 aa, unidentified
  REGION 1..151: note = Synthetic
MDWVWTLPFLMAAAQSIQAQIQLVQSGPELRKPGETVRISCKASGYPFTTAGLQWVQKMSGKGLKWIGWMNTQSEVPKYAEEFKGRIAFSLETAASTAYLQINNLKTEDTATYFCAKSVYFNWRYFDVWGAGTTVTVSSAKTTPPSVYPLA

SEQ ID NO: 9 - protein, 151 aa, unidentified
  REGION 1..151: note = Synthetic
MDWLWNLPFLMAAAQSIQAQIQLVQSGPELRKPGETVRISCKASGYPFTTAGLQWVQKMSGKGLKWIGWMNTQSEVPKYAEEFKGRIAFSLETAASTAYLQINNLKTEDTATYFCAKSVYFNWRYFDVWGAGTTVTVSSAKTTPPPVYPLA

SEQ ID NO: 10 - protein, 162 aa, unidentified
  REGION 1..162: note = Synthetic
MRAPAQFLGLLLLWTSASRCDIVMTQSPATLSVTPGDRVSLSCRASQSISDYLSWYQQRSHESPRLIIKYASQSISGIPSRFSGSGSGSDFTLSINSVEPEDVGVYYCQHGHSFPLTFGSGTKLELKRADAAPTVSIFPPSSEQLTSGGASVVCFLNNFYPK

SEQ ID NO: 11 - protein, 162 aa, unidentified
  REGION 1..162: note = Synthetic
MRAPAQLLGLLLFWTSASRCDIVMTQSPATLSVTPGDRVSLSCRASQSISDYLSWYQQRSHESPRLIIKYASQSISGIPSRFSGSGSGSDFTLNINSVEPEDVGVYYCQHGHSFPLTFGSGTKLELKRADAAPTVSIFPPSSEQLTSGGASVVCFLNNFYPK

SEQ ID NO: 12 - protein, 162 aa, unidentified
  REGION 1..162: note = Synthetic
MRSPAQFLGLLLFWTSASRCDIVMTQSPATLSVTPGDRVSLSCRASQSISDYLSWYQQRSHESPRLIIKYASQSISGIPSRFSGSGSGSDFTLSINSVEPEDVGVYYCQHGHSFPLTFGSGTKLELKRADAAPTVSIFPPSSEQLTSGGASVVCFLNNFYPK

SEQ ID NO: 13 - protein, 162 aa, unidentified
  REGION 1..162: note = Synthetic
MRSPAQFLGLLLFWTSASRCDIVMTQSPATLSVTPGDRVSLSCRASQSISDYLSWYQQRSHESPRLIIKYASQSISGIPSRFSGSGSGSDFTLSINSVEPEDVGVYYCQHGHSFPLTFGSGTKLELKRADAAPTVSIFPPSSEQLTSGGASVVCFLNNFYPR

SEQ ID NO: 14 - protein, 162 aa, unidentified
  REGION 1..162: note = Synthetic
MVSSAQFLGLLLFWTSASRCDIVMTQSPATLSVTPGDRVSLSCRASQSISDYLSWYQQRSHESPRLIIKYASQSISGIPSRFSGSGSGSDFTLSINSVEPEDVGVYYCQHGHSFPLTFGSGTKLELKRADAAPTVSIFPPSSEQLTSGGASVVCFLNNFYPK

SEQ ID NO: 15 - protein, 162 aa, unidentified
  REGION 1..162: note = Synthetic
MVSTAQFLGLLLFWTSASRCDIVMTQSPATLSVTPGDRVSLSCRASQSISDYLSWYQQRSHESPRLIIKYASQSISGIPSRFSGSGSGSDFTLSINSVEPEDVGVYYCQHGHSFPLTFGSGTKLELKRADAAPTVSIFPPSSEQLTSGGASVVCFLNNFYPR

SEQ ID NO: 16 - DNA, 453 bp, unidentified
  misc_feature 1..453: note = Synthetic
  source 1..453: mol_type = genomic DNA
atggaatggagctgtgtcatgctctttctcatggcagcagctcaaagtatccaagcacagatccagttggtgcagtctggacctgagctgaggaagcctggagagacagtcaggatctcctgcaaggcctctgggtatcccttcacaactgctggattgcagtgggtacagaagatgtcaggaaagggtttgaaatggattggctggatgaacacccagtctgaagtgccaaaatatgcagaagagttcaagggacggattgccttctctttggaaaccgctgccagtactgcatatttacagataaacaacctcaaaactgaggacacggcaacgtatttctgtgcgaaatcggtctattttaactggagatatttcgatgtctggggtgcagggaccacggtcaccgtctcctcagccaaaacgacacccccacccgtttatccactggcc

SEQ ID NO: 17 - DNA, 453 bp, unidentified
  misc_feature 1..453: note = Synthetic
  source 1..453: mol_type = genomic DNA
atgggatggagctgggtcatgctctttctcatggcagcagctcaaagtatccaagcacagatccagttggtgcagtctggacctgagctgaggaagcctggagagacagtcaggatctcctgcaaggcttctgggtatcccttcacaactgctggactgcagtgggtacagaagatgtcaggaaagggtttgaaatggattggctggatgaacacccagtctgaagtgccaaaatatgcagaagagttcaagggacggattgccttctctttggaaaccgctgccagtactgcatatttacagataaacaacctcaaaactgaggacacggcaacgtatttctgtgcgaaatcggtctattttaactggagatatttcgatgtctggggtgcagggaccacggtcaccgtctcctcagccaaaacgacacccccacccgtttatcccttggcc

SEQ ID NO: 18 - DNA, 453 bp, unidentified
  misc_feature 1..453: note = Synthetic
  source 1..453: mol_type = genomic DNA
atggaatgcagctgtgtaatgctctttctcatggcagcagctcaaagtatccaagcacagatccagttggtgcagtctggacctgagctgaggaagcctggagagacagtcaggatctcccgcaaggcttctgggtatcccttcacaactgctggattgcagtgggtacagaagatgtcaggaaagggtttgaaatggattggctggatgaacacccagtctgaagtgccaaaatatgcagaagagttcaagggacggattgccttctctttggaaaccgctgccagtactgcatatttacagataaacaacctcaaaactgaggacacggcaacgtatttctgtgcgaaatcggtctattttaactggagatatttcgatgtctggggtgcagggaccacggtcaccgtctcctcagccaaaacgacacccccatccgtcttccccctggca

SEQ ID NO: 19 - DNA, 453 bp, unidentified
  misc_feature 1..453: note = Synthetic
  source 1..453: mol_type = genomic DNA
atgggttgggtgtggaacttgctattcctcatggcagcagctcaaagtatccaagcacagatccagctggtgcagtctggacctgagctgaggaagcctggagagacagtcaggatctcctgcaaggcttctgggtatcccttcacaactgctggattgcagtgggtacagaagatgtcaggaaagggtttgaaatggattggctggatgaacacccagtctgaagtgccaaaatatgcagaagagttcaagggacggattgccttctctttggaaaccgctgccagtactgcatatttacagataaacaacctcaaaactgaggacacggcaacgtatttctgtgcgaaatcggtctattttaactggagatatttcgatgtctggggtgcagggaccacggtcaccgtctcctcagccaaaacgacacccccacccgtctatccactggtc

SEQ ID NO: 20 - DNA, 453 bp, unidentified
  misc_feature 1..453: note = Synthetic
  source 1..453: mol_type = genomic DNA
atggattgggtgtggaccttgccattcctcatggcagcagctcaaagtatccaagcacagatccagttggtgcagtctggacctgagctgaggaagcctggagagacagtcaggatctcctgcaaggcttctgggtatcccttcacaactgctggattgcagtgggtacagaagatgtcaggaaagggtttgaaatggattggctggatgaacacccagtctgaagtgccaaaatatgcagaagagttcaagggacggattgccttctctttggaaaccgctgccagtactgcatatttacagataaacaacctcaaaactgaggacacggcaacgtatttctgtgcgaaatcggtctattttaactggagatatttcgatgtctggggtgcagggaccacggtcaccgtctcctcagccaaaacgacacccccatctgtctatccactggcc

SEQ ID NO: 21 - DNA, 453 bp, unidentified
  misc_feature 1..453: note = Synthetic
  source 1..453: mol_type = genomic DNA
atgggttgggtgtggaacttgccattcctcatggcagcagctcaaagtatccaagcacagatccagttggtgcagtctggacctgagctgaggaagcctggagagacagtcaggatctcctgcaaggcttctgggtatcccttcacaactgctggattgcagtgggtacagaagatgtcaggaaagggtttgaaatggattggctggatgaacacccagtctgaagtaccaaaatatgcagaagagttcaagggacggattgccttctctttggaaaccgctgccagcactgcatatttacagataaacaacctcaaaactgaggacacggcaacgtatttctgtgcgaaatcggtctattttaactggagatatttcgatgtctggggtgcagggaccacggtcaccgtctcctcagccaaaacgacacccccacccgtctatccattggcc

SEQ ID NO: 22 - DNA, 453 bp, unidentified
  misc_feature 1..453: note = Synthetic
  source 1..453: mol_type = genomic DNA
atggattggctgtggaacttgccattcctcatggcagcagctcaaagtatccaagcacagatccagttggtgcagtctggacctgagctgaggaagcctggagagacagtcaggatctcctgcaaggcttctgggtatcccttcacaactgctggattgcagtgggtacagaagatgtcaggaaagggtttgaaatggattggctggatgaacacccagtctgaagtgccaaaatatgcagaagagttcaagggacggattgccttctctttggaaaccgctgccagtactgcatatttacagataaacaacctcaaaactgaggacacggcaacgtatttctgtgcgaaatcggtctattttaactggagatatttcgatgtctggggtgcagggaccacggtcaccgtctcctcagccaaaacgacacccccacccgtctatccactggcc

SEQ ID NO: 23 - DNA, 453 bp, unidentified
  misc_feature 1..453: note = Synthetic
  source 1..453: mol_type = genomic DNA
atgggttgggtgtggaccttgccattcctcatggcagcagctcaaagtatccaagcacagatccagttggtgcagtctggacctgagctgaggaagcctggagagacagtcaggatctcctgcaaggcttctgggtatcccttcacaactgctggattgcagtgggtacagaagatgtcaggaaagggtttgaaatggattggctggatgaacacccagtctgaagtgccaaaatatgcagaagagttcaagggacggattgccttctctttggaaaccgctgccagtactgcatatttacagataaacaacctcaaaactgaggacacggcgacgtatttctgtgcgaaatcggtctattttaactggagatatttcgatgtctggggtgcagggaccacggtcaccgtctcctcagccaaaacgacacccccacccgtctatcccctggtc

SEQ ID NO: 24 - DNA, 488 bp, unidentified
  misc_feature 1..488: note = Synthetic
  source 1..488: mol_type = genomic DNA
atgagggcccctgctcagtttcttgggcttttgcttctctggacttcagcctccagatgtgacattgtgatgactcagtctccagccaccctgtctgtgactccaggagatagagtctctctttcctgcagggccagccagagtattagcgactacttatcctggtatcaacaaagatctcatgagtctccaaggcttatcatcaaatatgcttcccaatccatctctgggatcccctccaggttcagtggcagtggatcagggtcagacttcactctcagtatcaacagtgtggaacctgaagatgttggagtgtattactgtcaacatggtcacagctttccgctcacgttcggttctgggaccaagctggagctgaaacgggctgatgctgcaccaactgtatccatcttcccaccatccagtgagcagttaacatctggaggtgcctcagtcgtgtgcttcttgaacaacttctaccccaaaga

SEQ ID NO: 25 - DNA, 486 bp, unidentified
  misc_feature 1..486: note = Synthetic
  source 1..486: mol_type = genomic DNA
atgaggtcccctgctcagttccttgggcttttgcttttctggacttcagcctccagatgtgacattgtgatgactcagtctccagccaccctgtctgtgactccaggagatagagtctctctttcctgcagggccagccagagtattagcgactacttatcctggtatcaacaaagatctcatgagtctccaaggcttatcatcaaatatgcttcccaatccatctctgggatcccctccaggttcagtggcagtggatcagggtcagacttcactctcagtatcaacagtgtggaacctgaagatgttggagtgtattactgtcaacatggtcacagctttccgctcacgttcggttctgggaccaagctggagctgaaacgggctgatgctgcaccaactgtatccatcttcccaccatccagtgagcagttaacatctggaggtgcctcagtcgtgtgcttcttgaacaacttctaccccaaa

SEQ ID NO: 26 - DNA, 488 bp, unidentified
  misc_feature 1..488: note = Synthetic
  source 1..488: mol_type = genomic DNA
atgaggtccccagctcagtttctggggcttttgcttttctggacttcagcctccagatgtgacattgtgatgactcagtctccagccaccctgtctgtgactccaggagatagagtctctctttcctgcagggccagccagagtattagcgactacttatcctggtatcaacaaagatctcatgagtctccaaggcttatcatcaaatatgcttcccaatccatctctgggatcccctccaggttcagtggcagtggatcagggtcagacttcactctcagtatcaacagtgtggaacctgaagatgttggagtgtattactgtcaacatggtcacagctttccgctcacgttcggttctgggaccaagctggagctgaaacgggctgatgctgcaccaactgtatccatcttcccaccatccagtgagcagttaacatctggaggtgcctcagtcgtgtgcttcttgaacaacttctaccccagaga

SEQ ID NO: 27 - DNA, 488 bp, unidentified
  misc_feature 1..488: note = Synthetic
  source 1..488: mol_type = genomic DNA
atgagggcccctgctcagctcctggggcttttgcttttctggacttcagcctccagatgtgacattgtgatgactcagtctccagccaccctgtctgtgactccaggagatagagtctctctttcctgcagggccagccagagtattagcgactacttatcctggtatcaacaaagatctcatgagtctccaaggcttatcatcaaatatgcttcccaatccatctctgggatcccctccaggttcagtggcagtggatcagggtcagacttcactctcaatatcaacagtgtggaacctgaagatgttggagtgtattactgtcaacatggtcacagctttccgctcacgttcggttctgggaccaagctggagctgaaacgggctgatgctgcaccaactgtatccatcttcccaccatccagtgagcagttaacatctggaggtgcctcagtcgtgtgcttcttgaacaacttctatcccaaaga

SEQ ID NO: 28 - DNA, 486 bp, unidentified
  misc_feature 1..486: note = Synthetic]
  source 1..486: mol_type = genomic DNA
atggtatcctcagctcagttccttggacttttgcttttctggacttcagcctccagatgtgacattgtgatgactcagtctccagccaccctgtctgtgactccaggagatagagtctctctttcctgcagggccagccagagtattagcgactacttatcctggtatcaacaaagatctcatgagtctccaaggcttatcatcaaatatgcttcccaatccatctctgggatcccctccaggttcagtggcagtggatcagggtcagacttcactctcagtatcaacagtgtggaacctgaagatgttggagtgtattactgtcaacatggtcacagctttccgctcacgttcggttctgggaccaagctggagctgaaacgggctgatgctgcaccaactgtatccatcttcccaccatccagtgagcagttaacatctggaggtgcctcagtcgtgtgcttcttgaacaacttctaccccaaa

SEQ ID NO: 29 - DNA, 488 bp, unidentified
  misc_feature 1..488: note = Synthetic
  source 1..488: mol_type = genomic DNA
atggtgtccacagctcagttccttggacttttgcttttctggacttcagcctccagatgtgacattgtgatgactcagtctccagccaccctgtctgtgactccaggagatagagtctctctttcctgcagggccagccagagtattagcgactacttatcctggtatcaacaaagatctcatgagtctccaaggcttatcatcaaatatgcttcccaatccatctctgggatcccctccaggttcagtggcagtggatcagggtcagacttcactctcagtatcaacagtgtggaacctgaagatgttggagtgtattactgtcaacatggtcacagctttccgctcacgttcggttctgggaccaagctggagctgaaacgggctgatgctgcaccaactgtatccatcttcccaccatccagtgagcagttaacatctggaggtgcctcagtcgtgtgcttcttgaacaacttctaccccagaga

SEQ ID NO: 30 - protein, 24 aa, unidentified
  REGION 1..24: note = Synthetic
EDYPPQKGCIPLPRGQTEKADHVD

SEQ ID NO: 31 - protein, 19 aa, unidentified
  REGION 1..19: note = Synthetic
QKGCIPLPRGQTEKADHVD

SEQ ID NO: 32 - protein, 15 aa, unidentified
  REGION 1..15: note = Synthetic
QKGCIPLPRGQTEKA

SEQ ID NO: 33 - protein, 106 aa, unidentified
  REGION 1..106: note = Synthetic
MNFGLSLVFLVLVLKGAQCEVQLVESGGGLVKPGGSLKLSCAASGFTFSDYYMYWVRQTPEKRLEWVATISDGGTYTYYPDSVKGRFTISRDNAKNNLYLQMNSLK

SEQ ID NO: 34 - protein, 147 aa, unidentified
  REGION 1..147: note = Synthetic
FLVLVLKGVQCEVQLVESGGGLVKPGGSLKLSCAASGFTFSDYYMYWVRQTPEKRLEWVATISDGGTYTYYPDSVKGRFTISRDNAKNNLYLQMNSLKSEDTAMYYCARGWVSTMVKLLSSFPYWGQGTLVTVSAAKTTPPSVYPLA

SEQ ID NO: 35 - protein, 155 aa, unidentified
  REGION 1..155: note = Synthetic
MDFGLSRVFLVLVLKGVQCEVQLVESGGGLVKPGGSLKLSCAASGFTFSDYYMYWVRQTPEKRLEWVATISDGGTYTYYPDSVKGRFTISRDNAKNNLYLQMNSLKSEDTAMYYCARGWVSTMVKLLSSFPYWGQGTLVTVSAAKTTPPSVYPLA

SEQ ID NO: 36 - protein, 155 aa, unidentified
  REGION 1..155: note = Synthetic
MDFGLSWVFLVLVLKGVQCEVQLVESGGGLVKPGGSLKLSCAASGFTFSDYYMYWVRQTPEKRLEWVATISDGGTYTYYPDSVKGRFTISRDNAKNNLYLQMNSLKSEDTAMYYCARGWVSTMVKLLSSFPYWGQGTLVTVSAAKTTPPSVYPLA

SEQ ID NO: 37 - protein, 149 aa, unidentified
  REGION 1..149: note = Synthetic
MAWISLIFSLLALSSGAISQAVVTQESALTTSPGETVTLTCRSSTGAVTTSNYANWVQEKPDHLFTGLVGGTNNRAPGVPARFSGSLIGDKAALTITGAQTEDEAIYFCALWYSNYWVFGGGTKLTVLGQPKSSPSVTLFPPSTEELSL

SEQ ID NO: 38 - protein, 149 aa, unidentified
  REGION 1..149: note = Synthetic
MAWISLIFSLLALSSGAISQAVVTQESALTTSPGETVTLTCRSSTGAVTTSNYANWVQEKPDHLFTGLIGGTSNRAPGVPARFSGSLIGDKAALTITGAQTEDEAIYFCALWYSNYWVFGGGTKLTVLGQPKSSPSVTLYPPSTKELSL

SEQ ID NO: 39 - protein, 149 aa, unidentified
  REGION 1..149: note = Synthetic
MAWTSLLLSLLALSSGAISQAVVTQESALTTSPGETVTLTCRSSTGAVTTSNYANWVQEKPDHLFTGLIGGTNNRAPGVPARFSGSLIGDKAALTITGAQTEDEAIYFCALWYSNYWVFGGGTKLTVLGQPKSSPSVTLCPPSSEKLSL

SEQ ID NO: 40 - protein, 149 aa, unidentified
  REGION 1..149: note = Synthetic
MAWTSLLFSLLALSSGAISQAVVTQESALTTSPGETVTLTCRSSTGAVTTSNYANWVQEKPDHLFTGLIGGTNNRAPGAPARFSGSLIGDKAALTITGAQTEDEAIYFCALWYSNYWVFGGGTKLTVLGQPKSSPSVTLCPPSTEKLSL

SEQ ID NO: 41 - protein, 149 aa, unidentified
  REGION 1..149: note = Synthetic
MAWIPLLFSLLALSSGAISQAVVTQESALTTSPGETVTLTCRSSTGAVTTSNYANWVQEKPDHLFTGLIGGTNNRAPGVPARFSGSLIGDKAALTIIGAQTEDEAIYFCALWYSNYWVFGGGTKLTVLGQPKSSPSVTLFPPSLEKLSL

SEQ ID NO: 42 - protein, 149 aa, unidentified
  REGION 1..149: note = Synthetic
MAWISLLLSLLALSSGAISQAVVTQESALTTSPGETVTLTCRSSTGAVTTSNYANWVQEKPDHLFTGLIGGTNNRAPGVPARFSGSLIGDKAALTITGAQTEDEAIYFCALWYSNYWVFGGGTKLTVLGQPKSSPSVTLFPPSTEELSL

SEQ ID NO: 43 - protein, 149 aa, unidentified
  REGION 1..149: note = Synthetic
MAWISLLFSLLALSSGAISQAVVTQESALTTSPGETVTLTCRSSTGAVTTSNYANWVQEKPDHLFTGLIGGTNNRAPGVPARFSGSLIGDKAALTITGAQTEDEAIYFCALWYSNYWVFGGGTKLTVLGQPKSSPSVTLFPPSTEKLSL

SEQ ID NO: 44 - DNA, 318 bp, unidentified
  misc_feature 1..318: note = Synthetic
  source 1..318: mol_type = genomic DNA
atgaacttcgggttgagcttggttttccttgtccttgttttaaaaggtgcccagtgtgaagtgcagctggtggagtctgggggaggcttagtgaagcctggagggtccctgaaactctcctgtgcagcctctggattcactttcagtgactattacatgtattgggttcgccagactccggaaaagaggctggagtgggtcgcaaccattagtgatggtggtacttacacctactatccagacagtgtgaaggggcgattcaccatctccagagacaatgccaagaacaacctttacctgcaaatgaacagtctgaag

SEQ ID NO: 45 - DNA, 465 bp, unidentified
  misc_feature 1..465: note = Synthetic
  source 1..465: mol_type = genomic DNA
atggacttcgggttgagctgggttttccttgtccttgttttaaaaggtgtccagtgtgaagtgcagctggtggagtctgggggaggcttagtgaagcctggagggtccctgaaactctcctgtgcagcctctggattcactttcagtgactattacatgtattgggttcgccagactccggaaaagaggctggagtgggtcgcaaccattagtgatggtggtacttacacctactatccagacagtgtgaaggggcgattcaccatctccagagacaatgccaagaacaacctttacctgcaaatgaacagtctgaagtctgaggacacagccatgtattactgtgcaagaggatgggtttctactatggttaaacttctttcctcctttccttactggggccaagggactctggtcactgtctctgcagccaaaacgacacccccatctgtctatccactggcc

SEQ ID NO: 46 - DNA, 465 bp, unidentified
  misc_feature 1..465: note = Synthetic
  source 1..465: mol_type = genomic DNA
atggacttcgggctgagcagggttttccttgtccttgttttaaaaggtgtccagtgtgaagtgcagctggtggagtctgggggaggcttagtgaagcctggagggtccctgaaactctcctgtgcagcctctggattcactttcagtgactattacatgtattgggttcgccagactccggaaaagaggctggagtgggtcgcaaccattagtgatggtggtacttacacctactatccagacagtgtgaaggggcgattcaccatctccagagacaatgccaagaacaacctttacctgcaaatgaacagtctgaagtctgaggacacagccatgtattactgtgcaagaggatgggtttctactatggttaaacttctttcctcctttccttactggggccaagggactctggtcactgtctctgcagccaaaacgacacccccatctgtctatccactggcc

SEQ ID NO: 47 - DNA, 465 bp, unidentified
  misc_feature 1..465: note = Synthetic
  source 1..465: mol_type = genomic DNA
atggacttcgggctgagctgggttttccttgtccttgttttaaaaggtgtccagtgtgaagtgcagctggtggagtctgggggaggcttagtgaagcctggagggtccctgaaactctcctgtgcagcctctggattcactttcagtgactattacatgtattgggttcgccagactccggaaaagaggctggagtgggtcgcaaccattagtgatggtggtacttacacctactatccagacagtgtgaaggggcgattcaccatctccagagacaatgccaagaacaacctttacctgcaaatgaacagtctgaagtctgaggacacagccatgtattactgtgcaagaggatgggtttctactatggttaaacttctttcctcctttccttactggggccaagggactctggtcactgtctctgcagccaaaacgacacccccatctgtctatccactggcc

SEQ ID NO: 48 - DNA, 443 bp, unidentified
  misc_feature 1..443: note = Synthetic
  source 1..443: mol_type = genomic DNA
ttttccttgtccttgttttaaaaggtgtccagtgtgaagtgcagctggtggagtctgggggaggcttagtgaagcctggagggtccctgaaactctcctgtgcagcctctggattcactttcagtgactattacatgtattgggttcgccagactccggaaaagaggctggagtgggtcgcaaccattagtgatggtggtacttacacctactatccagacagtgtgaaggggcgattcaccatctccagagacaatgccaagaacaacctttacctgcaaatgaacagtctgaagtctgaggacacagccatgtattactgtgcaagaggatgggtttctactatggttaaacttctttcctcctttccttactggggccaagggactctggtcactgtctctgcagccaaaacgacacccccatctgtctatccactggcc

SEQ ID NO: 49 - DNA, 465 bp, unidentified; identical to SEQ ID NO: 47
  misc_feature 1..465: note = Synthetic
  source 1..465: mol_type = genomic DNA

SEQ ID NO: 50 - DNA, 449 bp, unidentified
  misc_feature 1..449: note = Synthetic
  source 1..449: mol_type = genomic DNA
atggcctggatttctcttatattctctctcctggctctcagctcaggggccatttcccaggctgttgtgactcaggaatctgcactcaccacatcacctggtgaaacagtcacactcacttgtcgctcaagtactggggctgttacaactagtaactatgccaactgggtccaagaaaaaccagatcatttattcactggtctagtaggtggtaccaacaaccgagctccaggtgttcctgccagattctcaggctccctgattggagacaaggctgccctcaccatcacaggggcacagactgaggatgaggcaatatatttctgtgctctatggtacagcaattattgggtgttcggtggaggaaccaaactgactgtcctaggccagcccaagtcttcgccatcagtcaccctgttcccaccctccactgaagagctaagcttggg

SEQ ID NO: 51 - DNA, 449 bp, unidentified
  misc_feature 1..449: note = Synthetic
  source 1..449: mol_type = genomic DNA
atggcctggacttcactcttactctctctcctggctctcagctcaggggccatttcccaggctgttgtgactcaggaatctgcactcaccacatcacctggtgaaacagtcacactcacttgtcgctcaagtactggggctgttacaactagtaactatgccaactgggtccaagaaaaaccagatcatttattcactggtctaataggtggtaccaacaaccgagctccaggtgttcctgccagattctcaggctccctgattggagacaaggctgccctcaccatcacaggggcacagactgaggatgaggcaatatatttctgtgctctatggtacagcaattattgggtgttcggtggaggaaccaaactgactgtcctaggccagcccaagtcttcgccatcagtcaccctgtgcccgccctcctcagagaagctaagcttggg

SEQ ID NO: 52 - DNA, 449 bp, unidentified
  misc_feature 1..449: note = Synthetic
  source 1..449: mol_type = genomic DNA
atggcctggattcctcttttattctctctcctggctctcagctcaggggccatttcccaggctgttgtgactcaggaatctgcactcaccacatcacctggtgaaacagtcacactcacttgtcgctcaagtactggggctgttacaactagtaactatgccaactgggtccaagaaaaaccagatcatttattcactggtctaataggtggtaccaacaaccgagctccaggtgttcctgccagattctcaggctccctgattggagacaaggctgccctcaccatcataggggcacagactgaggatgaggcaatatatttctgtgctctatggtacagcaattattgggtgttcggtggaggaaccaaactgactgtcctaggccagcccaagtcttcgccatcagtcaccctgttcccgccctccttagaaaagcttagcttggg

SEQ ID NO: 53 - DNA, 449 bp, unidentified
  misc_feature 1..449: note = Synthetic
  source 1..449: mol_type = genomic DNA
atggcctggatttcacttttactctctctcctggctctcagctcaggggccatttcccaggctgttgtgactcaggaatctgcactcaccacatcacctggtgaaacagtcacactcacttgtcgctcaagtactggggctgttacaactagtaactatgccaactgggtccaagaaaaaccagatcatttattcactggtctaataggtggtaccaacaaccgagctccaggtgttcctgccagattctcaggctccctgattggagacaaggctgccctcaccatcacaggggcacagactgaggatgaggcaatatatttctgtgctctatggtacagcaattattgggtgttcggtggaggaaccaaactgactgtcctaggccagcccaagtcttcgccatcagtcaccctgtttccaccctccacagaagagctaagcttggg

SEQ ID NO: 54 - DNA, 449 bp, unidentified
  misc_feature 1..449: note = Synthetic
  source 1..449: mol_type = genomic DNA
atggcctggatttcacttatcttctctctcctggctctcagctcaggggccatttcccaggctgttgtgactcaggaatctgcactcaccacatcacctggtgaaacagtcacactcacttgtcgctcaagtactggggctgttacaactagtaactatgccaactgggtccaagaaaaaccagatcatttattcactggtctaataggtggtaccagcaaccgagctccaggtgttcctgccagattctcaggctccctgattggagacaaggctgccctcaccatcacaggggcacagactgaggatgaggcaatatatttctgtgctctatggtacagcaattattgggtgttcggtggaggaaccaaactgactgtcctaggccagcccaagtcttcgccatcagtcaccctgtacccgccctctacaaaggagcttagcttggg

SEQ ID NO: 55 - DNA, 449 bp, unidentified
  misc_feature 1..449: note = Synthetic
  source 1..449: mol_type = genomic DNA
atggcctggacttctctcttattctctctcctggctctcagctcaggggccatttcccaggctgttgtgactcaggaatctgcactcaccacatcacctggtgaaacagtcacactcacttgtcgctcaagtactggggctgttacaactagtaactatgccaactgggtccaagaaaaaccagatcatttattcactggtctaataggtggtaccaacaaccgagctccaggtgctcctgccagattctcaggctccctgattggagacaaggctgccctcaccatcacaggggcacagactgaggatgaggcaatatatttctgtgctctatggtacagcaattattgggtgttcggtggaggaaccaaactgactgtcctaggccagcccaagtcttcgccatcagtcaccctgtgcccgccctctacagaaaagctaagcttggg

SEQ ID NO: 56 - DNA, 708 bp, unidentified
  misc_feature 1..708: note = Synthetic
  source 1..708: mol_type = genomic DNA
atggtcagctctgctcaatttctcggactccttcttctgtgctttcaaggaacacgctgcgatattgtgatgacccagtcccccgccaccctgtccgtgactccgggcgaccgggtgtccctgtcgtgccgggcatcacagagcatctccgactacctgtcgtggtaccagcagagatcacacgagagccctcgcctgatcatcaaatacgccagccagtcaatctccggcatcccctcgcggttctccgggtccggttccggctccgacttcacactgtccattaactccgtggaacctgaggacgtgggagtgtactactgtcaacacggccattcgttcccgctgactttcgggtcgggaaccaagctggaattgaagagggcggacgcggcccctaccgtgtcaattttcccaccgagctccgaacagctcaccagcggcggtgcctcggtcgtgtgcttcctcaacaacttctatccaaaagacattaacgtcaagtggaagatcgatggatcggagagacagaacggagtgctgaacagctggactgatcaggactccaaggattcgacctactccatgagctccactctgaccctgaccaaggacgaatacgagcggcacaattcctacacttgcgaagccacccacaagacctcaacgtcccccatcgtgaagtccttcaaccgcaacgagtgttgataa

SEQ ID NO: 57 - protein, 234 aa, unidentified
  REGION 1..234: note = Synthetic
MVSSAQFLGLLLLCFQGTRCDIVMTQSPATLSVTPGDRVSLSCRASQSISDYLSWYQQRSHESPRLIIKYASQSISGIPSRFSGSGSGSDFTLSINSVEPEDVGVYYCQHGHSFPLTFGSGTKLELKRADAAPTVSIFPPSSEQLTSGGASVVCFLNNFYPKDINVKWKIDGSERQNGVLNSWTDQDSKDSTYSMSSTLTLTKDEYERHNSYTCEATHKTSTSPIVKSFNRNEC

SEQ ID NO: 58 - DNA, 2201 bp, unidentified
  misc_feature 1..2201: note = Synthetic
  source 1..2201: mol_type = genomic DNA
atgggctggaccctcgtgttcctgttcctgctgagcgtgacggcgggcgtgcactcccaaatccagcttgtgcagtccggacccgagctcaggaagccgggcgaaactgtgcgcatcagctgcaaggcttcagggtaccctttcaccaccgccgggctgcaatgggtgcagaagatgtccgggaagggtctgaagtggatcggatggatgaacacccagtccgaagtgcctaaatacgccgaagaattcaagggccgcattgcgttcagcctggagacagccgcctcgaccgcgtaccttcagatcaacaatctcaagactgaggacactgccacctacttctgtgccaagagcgtgtacttcaactggagatacttcgacgtgtggggcgccggaaccaccgtgaccgtgtccagcgccaagactaccgccccgagcgtgtaccctctggcgccagtgtgcggcgacacgactggcagctcggtgaccttgggctgcctcgtgaagggttacttccccgagcccgtgactctgacttggaactcgggctcactgtcgtccggagtgcataccttcccggctgtgctgcaaagcgacctctataccttgtcatcgtccgtgactgtgacctcctccacctggccgtcccagagcatcacctgtaatgtcgcccaccctgcttcatcgactaaggtcgacaagaagatcgagcccagaggacctaccatcaagccctgcccgccctgcaaatgcccggccccaaacttgctgggagggccttccgtgttcatcttccctccgaaaatcaaggacgtgctgatgatctccctgagcccaattgtcacttgcgtggtggtggatgtgtccgaagatgacccagatgtgcagatttcatggttcgtgaacaacgtcgaagtccataccgcacagacccagacccaccgcgaggattacaactcgacgctgcgcgtcgtcagcgccctgccgattcagcaccaggattggatgagcggaaaggaattcaagtgcaaagtcaacaacaaggaccttccggcgccgatcgaacggaccatctcgaagcctaagggatcagtgcgggcgcctcaggtctacgtgctcccgcctccggaagaggaaatgaccaagaaacaagtcaccctgacttgcatggtcaccgacttcatgcctgaggacatctatgtggagtggactaacaacggaaagactgaactgaactacaaaaacaccgaaccagtgctggactctgacggctcctacttcatgtactcgaagctgcgggtggagaagaaaaactgggtggaacgaaactcctactcgtgttccgtggtgcacgagggtctgcacaaccaccataccaccaagtccttctcccggacccccggaaagggatccgccgggggatccggaggggactccgaagtgcaactggtggagtcgggtggcggactcgtgaagcccggggggtcattgaagctttcctgtgctgcctccggtttcactttctccgactattacatgtactgggtcagacagaccccggagaagcggctcgaatgggtggccaccatttcggacggtggaacctacacttactaccctgactccgtcaagggccggtttactatctcccgcgacaacgcgaagaacaatctgtacctccaaatgaactccctgaagtccgaggacaccgccatgtactattgcgcaaggggatgggtcagcactatggtcaagctgctgtcatccttcccttactggggacagggaacccttgtgactgtgtcagccggtggcggggggtcgggcggcggcggttccggtggagggggatcccaggccgtcgtgacccaagagtcggctctgactacttcacccggagaaaccgtgaccctgacatgccgctcctccactggcgcagtgaccacgagcaattacgccaactgggtgcaggaaaagcccgatcacctgttcactggactcattgggggaaccaacaaccgggcgccgggcgtgcccgctcggtttagcggctccctgattggagacaaggccgccctgactatcaccggagcccagaccgaagatgaagccatctacttttgcgcactctggtactctaactactgggtgtttggcggcggaaccaagctgactgtgctcggacagccgaagtgataaaa

SEQ ID NO: 59 - protein, 731 aa, unidentified
  REGION 1..731: note = Synthetic
MGWTLVFLFLLSVTAGVHSQIQLVQSGPELRKPGETVRISCKASGYPFTTAGLQWVQKMSGKGLKWIGWMNTQSEVPKYAEEFKGRIAFSLETAASTAYLQINNLKTEDTATYFCAKSVYFNWRYFDVWGAGTTVTVSSAKTTAPSVYPLAPVCGDTTGSSVTLGCLVKGYFPEPVTLTWNSGSLSSGVHTFPAVLQSDLYTLSSSVTVTSSTWPSQSITCNVAHPASSTKVDKKIEPRGPTIKPCPPCKCPAPNLLGGPSVFIFPPKIKDVLMISLSPIVTCVVVDVSEDDPDVQISWFVNNVEVHTAQTQTHREDYNSTLRVVSALPIQHQDWMSGKEFKCKVNNKDLPAPIERTISKPKGSVRAPQVYVLPPPEEEMTKKQVTLTCMVTDFMPEDIYVEWTNNGKTELNYKNTEPVLDSDGSYFMYSKLRVEKKNWVERNSYSCSVVHEGLHNHHTTKSFSRTPGKGSAGGSGGDSEVQLVESGGGLVKPGGSLKLSCAASGFTFSDYYMYWVRQTPEKRLEWVATISDGGTYTYYPDSVKGRFTISRDNAKNNLYLQMNSLKSEDTAMYYCARGWVSTMVKLLSSFPYWGQGTLVTVSAGGGGSGGGGSGGGGSQAVVTQESALTTSPGETVTLTCRSSTGAVTTSNYANWVQEKPDHLFTGLIGGTNNRAPGVPARFSGSLIGDKAALTITGAQTEDEAIYFCALWYSNYWVFGGGTKLTVLGQPK

SEQ ID NO: 60 - protein, 8 aa, unidentified
  REGION 1..8: note = Synthetic
GYPFTTAG

SEQ ID NO: 61 - protein, 8 aa, Unknown
MNTQSEVP

SEQ ID NO: 62 - protein, 13 aa, Unknown
AKSVYFNWRYFDV

SEQ ID NO: 63 - protein, 6 aa, Unknown
QSISDY

SEQ ID NO: 64 - protein, 9 aa, Unknown
QHGHSFPLT

SEQ ID NO: 65 - protein, 8 aa, Unknown
GFTFSDYY

SEQ ID NO: 66 - protein, 8 aa, Unknown
ISDGGTYT

SEQ ID NO: 67 - protein, 17 aa, Unknown
ARGWVSTMVKLLSSFPY

SEQ ID NO: 68 - protein, 9 aa, Unknown
TGAVTTSNY

SEQ ID NO: 69 - protein, 9 aa, Unknown
ALWYSNYWV